European Patent Specification EP 3 986 144 B1, published September 24, 2025. Title: CROSS-LINKED MILK PROTEIN CO-PRECIPITATE. Applicant: Novozymes A/S. The sequence listing filed with the application follows.

SEQUENCE LISTING (2 sequences)

SEQ ID NO: 1 - protein, 331 aa, Streptomyces mobaraensis
DSDDRVTPPAEPLDRMPDPYRPSYGRAETVVNNYIRKWQQVYSHRDGRKQQMTEEQREWLSYGCVGVTWVNSGQYPTNRLAFASFDEDRFKNELKNGRPRSGETRAEFEGRVAKESFDEEKGFQRAREVASVMNRALENAHDESAYLDNLKKELANGNDALRNEDARSPFYSALRNTPSFKERNGGNHDPSRMKAVIYSKHFWSGQDRSSSADKRKYGDPDAFRPAPGTGLVDMSRDRNIPRSPTSPGEGFVNFDYGWFGAQTEADADKTVWTHGNHYHAPNGSLGAMHVYESKFRNWSEGYSDFDRGAYVITFIPKSWNTAPDKVKQGWP

SEQ ID NO: 2 - protein, 418 aa, Streptomyces lydicus
MYKRRSLLAFATVSAAIFTAGVMPSVSHAASGGDGEREGSYAETHGLTAEDVKNINALNKRALNAGQPGNSLAELPPSVSALFRAPDAADERVTPPAEPLNRMPDAYRAYGGRATTVVNNYIRKWQQVYSHRDGIQQQMTEEQREKLSYGCVGITWVNSGPYPTNKLAFAFFDENKYKSDLENSRPRPNETQAEFEGRIVKDSFDEGKGFKRARDVASVMNKALDSAHDEGTYIDNLKTELANKNDALRYEDGRSNFYSALRNTPSFKERDGGNYDPSKMKAVVYSKHFWSGQDQRGSSDKRKYGDPDAFRPDQGTGLVDMSKDRNIPRSPAQPGESWVNFDYGWFGAQTESDADKTIWTHANHYHAPNGGLGPMNVYESKFRNWSAGYADFDRGTYVITFIPKSWNTAPAEVKQGWS